European Patent Specification EP 4 001 306 B1, published August 27, 2025. Title: HUMANIZED ANTI-VEGF MONOCLONAL ANTIBODY. Applicant: SinoCellTech Ltd. The sequence listing filed with the application follows.

SEQUENCE LISTING (98 sequences)

SEQ ID NO: 1 - protein, 191 aa, Homo sapiens
MNFLLSWVHWSLALLLYLHHAKWSQAAPMAEGGGQNHHEVVKFMDVYQRSYCHPIETLVDIFQEYPDEIEYIFKPSCVPLMRCGGCCNDEGLECVPTEESNITMQIMRIKPHQGQHIGEMSFLQHNKCECRPKKDRARQEKKSVRGKGKGQKRKRKKSRYKSWSVYVGARCCLMPWSLPGPHPCGPCSERR

SEQ ID NO: 2 - DNA, 54 bp, Artificial Sequence
  Nucleotide sequence of the linker used in the construction of the phage antibody library for the linkage of the rabbit antibody scFv
tctagtggtggcggtggttcgggcggtggtggaggtggtagttctagatcttcc

SEQ ID NO: 3 - DNA, 732 bp, Artificial Sequence
  Nucleotide sequence of rabbit antibody scFv used in the construction of antibody VEGF165-R859
gatgtcgtgatgacccagactgcagcctccgtgtctgaacctgtgggaggcacagtcaccatcaagtgccaggccagtcagagcattaggagttggttatcctggtatcagcagaaaccagggcagcctcccaagctcctgatctatcaggcatccaaattggcatctggggtcccatcgcggttcaaaggcagtggatatgggacagagttcactctcaccatcagcgacctggagtgtgccgatgctgccacttactactgtcaaaacaattattcttttagtaaagatggtggtgctttcggcggagggaccgaggtggtcgtcaaatctagtggtggcggtggttcgggcggtggtggaggtggtagttctagatcttcccagtcggtggaggagtccgggggtcgcctggtcacgcctgggacacccctgacactcacctgccaagtctctggattctccctcaacatctacgacatgacctgggtccgccaggctccagggaaggggctggaatggatcggaatcattgcgcctgatgatagcgcatactacgcgaactgggcgaaaggccgattcaccatctccaaaacctcgaccacggtggatctgaaaatgaccagtccgacaaccgaggacacggccacctatttctgtgccagaaatgcctatagtagtggctggggtggggacttgtggggcccaggcaccctggtcactgtctcttca

SEQ ID NO: 4 - DNA, 738 bp, Artificial Sequence
  Nucleotide sequence of the rabbit antibody scFv used in the construction of antibody VEGF165-R988
gagctcgatctgacccagactccatcccccgtgtctgcggctgttggaggcacagtcaccatcaattgccagtccagtcagactatttatgctaacaggcgcttagcctggtatcaacagaaaccagggcagcctcccaagctcctgatctatggtgcatccactctggcatctggggtcccatcgcggttcaaaggcagtggatctgggacacagttcactctcaccatcagcggcgtgcagtgtgacgatgctgccacttactactgtgcaggctataaaagttatgatggtgatgatgttggtttcggcggagggaccgaggtggtcgtcaaatctagtggtggcggtggttcgggcggtggtggaggtggtagttctagatcttcccagtcggtggaggagtccgggggtcgcctggtaacgcctgggacacccctgacactcacctgcacagtctctggaatcgacctcagtagctatgcaataagctgggtccgccaggctccagggaaggggctggaatacatcggatacatttggaatgctggtaacacctactacgcgagctgggcaaaaggccgattcaccatctccaaaacctcgaccacggtggatctgaaaatcaccagtccgacaaccgaggacacggccacctatttctgtgccagaggaacattaggggactacaatggcatggacccctggggcccagggaccctcgtcaccgtctcttca

SEQ ID NO: 5 - DNA, 738 bp, Artificial Sequence
  Nucleotide sequence of the rabbit antibody scFv used in the construction of  antibody VEGF165-R613
gagctcgtgatgacccagactccatcccccgtgtctgcggctgttggaggcacagtcaccatcaattgccagtccagtcagagtgtttatagtaacaaccggttagcctggtatcagcagaaaccagggcagcctcccaagctcctgatctatggtgcatccactctggcatctggggtcccatcgcggttcaaaggcagtggatctgggacacagttcactctcaccatcagcgacgtgcagtgtgacgatgctgccacttactactgtgcaggctataaaagttatgatggtgatgatgttggtttcggcggagggaccgaggtggtggtcaaatctagtggtggcggtggttcgggcggtggtggaggtggtagttctagatcttcccagtcggtggaggagtccgggggtcgcctggtcacgcctgggacacccctgacactcacctgcacagtctctggaatcgacctcagtagctatgcaataagctgggtccgccaggctccagggaaggggctggaatacatcggatacatttggagtactgataacacctactatgcgagctgggcaaaaggccgattcaccatctccgaggcctcgaccacggtggatctgaaaatcaccagcccgacaaccgaggacacggccacctatttctgtgccagaggaacgttaggggactacaatggcatggacccctggggcccagggaccctcgtcaccgtctcttca

SEQ ID NO: 6 - DNA, 738 bp, Artificial Sequence
  Nucleotide sequence of the rabbit antibody scFv used in the construction of  antibody VEGF165-R812
gagctcgtgctgacccagactccagcctccgtggaggcagctgtgggaggcacagtcaccatcaagtgccaggccagtcagagcattaatagttggttatcctggtatcagcagaaaccagggcagcgtcccaagctcctgatctaccaggcatccaaactggcatctggggtcccatcgcggttcaaaggcagtggatctgggacagagtacactctcaccatcagcgacctggagtgtgccgatgctgccacttattactgccagaacaatcttggtggtggtgatggtagttatggtcttcctttcggcggagggaccgaggtggtggtcaaatctagtggtggcggtggttcgggcggtggtggaggtggtagttctagatcttcccagtcgttggaggagtccgggggtcgcctggtaacgcctggaggctccctgacactcacctgcacagcctctggattcgacctcggtatctatgaaataacctgggtccgccaggctccagggaaggggctggaatggatcggagtcatttatggtgatggtgacacagtctacgcgaactgggcgaaaggccgattcaccatctccaaaacctcgaccacggtggatctgaaaatctccagtccgacaaccgaggacacggccacctatttctgtgccagaaatggctatactactggctggggtggggacttgtggggcccaggcaccctggtcactgtctcttca

SEQ ID NO: 7 - DNA, 348 bp, Oryctolagus cuniculus f. domesticus
cagtcggtggaggagtccgggggtcgcctggtaacgcctgggacacccctgacactcacctgcacagtctctggaatcgacctcagtagctatgcaataagctgggtccgccaggctccagggaaggggctggaatacatcggatacatttggaatgctggtaacacctactacgcgagctgggcaaaaggccgattcaccatctccaaaacctcgaccacggtggatctgaaaatcaccagtccgacaaccgaggacacggccacctatttctgtgccagaggaacattaggggactacaatggcatggacccctggggcccagggaccctcgtcaccgtctcttca

SEQ ID NO: 8 - DNA, 336 bp, Oryctolagus cuniculus f. domesticus
gagctcgatctgacccagactccatcccccgtgtctgcggctgttggaggcacagtcaccatcaattgccagtccagtcagactatttatgctaacaggcgcttagcctggtatcaacagaaaccagggcagcctcccaagctcctgatctatggtgcatccactctggcatctggggtcccatcgcggttcaaaggcagtggatctgggacacagttcactctcaccatcagcggcgtgcagtgtgacgatgctgccacttactactgtgcaggctataaaagttatgatggtgatgatgttggtttcggcggagggaccgaggtggtcgtcaaa

SEQ ID NO: 9 - DNA, 972 bp, Oryctolagus cuniculus f. domesticus
ggtcaacctaaggctccgtcagtcttcccactggccccctgctgcggggacacacccagctccacggtgaccctgggctgcctggtcaaaggctacctcccggagccagtgaccgtgacctggaactcgggcaccctcaccaatggggtacgcaccttcccgtccgtccggcagtcctcaggcctctactcgctgagcagcgtggtgagcgtgacctcaagcagccagcccgtcacctgcaacgtggcccacccagccaccaacaccaaagtggacaagaccgttgcgccctcgacatgcagcaagcccacgtgcccaccccctgaactcctggggggaccgtctgtcttcatcttccccccaaaacccaaggacaccctcatgatctcacgcacccccgaggtcacatgcgtggtggtggacgtgagccaggatgaccccgaggtgcagttcacatggtacataaacaacgagcaggtgcgcaccgcccggccgccgctacgggagcagcagttcaacagcacgatccgcgtggtcagcaccctccccatcgcgcaccaggactggctgaggggcaaggagttcaagtgcaaagtccacaacaaggcactcccggcccccatcgagaaaaccatctccaaagccagagggcagcccctggagccgaaggtctacaccatgggccctccccgggaggagctgagcagcaggtcggtcagcctgacctgcatgatcaacggcttctacccttccgacatctcggtggagtgggagaagaacgggaaggcagaggacaactacaagaccacgccggccgtgctggacagcgacggctcctacttcctctacagcaagctctcagtgcccacgagtgagtggcagcggggcgacgtcttcacctgctccgtgatgcacgaggccttgcacaaccactacacgcagaagtccatctcccgctctccgggtaaataa

SEQ ID NO: 10 - DNA, 315 bp, Oryctolagus cuniculus f. domesticus
ggggatccagttgcacctactgtcctcatcttcccaccagctgctgatcaggtggcaactggaacagtcaccatcgtgtgtgtggcgaataaatactttcccgatgtcaccgtcacctgggaggtggatggcaccacccaaacaactggcatcgagaacagtaaaacaccgcagaattctgcagattgtacctacaacctcagcagcactctgacactgaccagcacacagtacaacagccacaaagagtacacctgcaaggtgacccagggcacgacctcagtcgtccagagcttcaataggggtgactgttaa

SEQ ID NO: 11 - protein, 116 aa, Oryctolagus cuniculus f. domesticus
QSVEESGGRLVTPGTPLTLTCTVSGIDLSSYAISWVRQAPGKGLEYIGYIWNAGNTYYASWAKGRFTISKTSTTVDLKITSPTTEDTATYFCARGTLGDYNGMDPWGPGTLVTVSS

SEQ ID NO: 12 - protein, 112 aa, Oryctolagus cuniculus f. domesticus
ELDLTQTPSPVSAAVGGTVTINCQSSQTIYANRRLAWYQQKPGQPPKLLIYGASTLASGVPSRFKGSGSGTQFTLTISGVQCDDAATYYCAGYKSYDGDDVGFGGGTEVVVK

SEQ ID NO: 13 - protein, 13 aa, Oryctolagus cuniculus f. domesticus
QSSQTIYANRRLA

SEQ ID NO: 14 - protein, 7 aa, Oryctolagus cuniculus f. domesticus
GASTLAS

SEQ ID NO: 15 - protein, 12 aa, Oryctolagus cuniculus f. domesticus
AGYKSYDGDDVG

SEQ ID NO: 16 - protein, 10 aa, Oryctolagus cuniculus f. domesticus
GIDLSSYAIS

SEQ ID NO: 17 - protein, 16 aa, Oryctolagus cuniculus f. domesticus
YIWNAGNTYYASWAKG

SEQ ID NO: 18 - protein, 13 aa, Oryctolagus cuniculus f. domesticus
ARGTLGDYNGMDP

SEQ ID NO: 19 - DNA, 1404 bp, Artificial sequence
  Nucleotide sequence of the humanized antibody VEGF165-H988-10 heavy chain containing signal peptide
atgggctggtccctgattctgctgttcctggtggctgtggctaccagggtgctgagtcagtctgtccaggagtctggacctggactggtgaagccatctgagaccctgtccctgacttgtactgtgtctggcattgacctgtcctcctatgccatctcctgggtgagacaacctcctggcaagggattggaatacattggctacatctggaatgctggcaacacctactatgcctcctgggctaagggcagggtgaccatctctgtggacaccagcaagaaccaggtggacctgaaactgtcctctgtgacagcagcagacacagcagtctacttctgtgccaggggcaccctgggagactacaatgggatggacccatggggacctggcaccctggtgacagtgtccagcgctagcaccaagggcccatcggtcttccccctggcaccctcctccaagagcacctctgggggcacagcggccctgggctgcctggtcaaggactacttccccgaaccggtgacggtgtcgtggaactcaggcgccctgaccagcggcgtgcacaccttcccggctgtcctacagtcctcaggactctactccctcagcagcgtggtgaccgtgccctccagcagcttgggcacccagacctacatctgcaacgtgaatcacaagcccagcaacaccaaggtggacaagaaagttgagcccaaatcttgtgacaaaactcacacatgcccaccgtgcccagcacctgaactcctggggggaccgtcagtcttcctcttccccccaaaacccaaggacaccctcatgatctcccggacccctgaggtcacgtgcgtggtggtggacgtgagccacgaagaccccgaggtcaagttcaactggtacgtggacggcgtggaggtgcataatgccaagacaaagccgcgggaggagcagtacaacagcacgtaccgtgtggtcagcgtcctcaccgtcctgcaccaggactggctgaatggcaaggagtacaagtgcaaggtctccaacaaagccctcccagcccccatcgagaaaaccatctccaaagccaaagggcagccccgagaaccacaggtgtacaccctgcccccatcccgggatgagctgaccaagaaccaggtcagcctgacctgcctggtcaaaggcttctatcccagcgacatcgccgtggagtgggagagcaatgggcagccggagaacaactacaagaccacgcctcccgtgctggactccgacggctccttcttcctctacagcaagctcaccgtggacaagagcaggtggcagcaggggaacgtcttctcatgctccgtgatgcatgaggctctgcacaaccactacacgcagaagagcctctccctgtctccgggtaaatga

SEQ ID NO: 20 - DNA, 717 bp, Artificial sequence
  Nucleotide sequence of humanized antibody VEGF165-H988-10 light chain containing signal peptide
atgggctggtcctgtatcatcctgttcctggtggctacagccacaggagtgcatagtgaactccaacttacccagagcccatcctccctgtctgcctctgtgggagacagggtgaccatcacttgtcagtccagccagaccatctatgccaacaggagactggcttggtatcaacagaagcctggcaaggtgccaaaactgctgatttatggagccagcaccctggcatctggagtgccaagcaggttcaagggctctggctctggcacagacttcaccctgaccatctcctccctccaacctgaggatgtggctacctactactgtgctggctacaagtcctatgatggagatgatgtgggctttggaggaggcaccaaggtggagattaagcgtacggtggctgcaccatctgtcttcatcttcccgccatctgatgagcagttgaaatctggaactgcctctgttgtgtgcctgctgaataacttctatcccagagaggccaaagtacagtggaaggtggataacgccctccaatcgggtaactcccaggagagtgtcacagagcaggacagcaaggacagcacctacagcctcagcagcaccctgacgctgagcaaagcagactacgagaaacacaaagtctacgcctgcgaagtcacccatcagggcctgagctcgcccgtcacaaagagcttcaacaggggagagtgttag

SEQ ID NO: 21 - protein, 467 aa, Artificial sequence
  Amino acid sequence of the heavy chain of humanized antibody VEGF165-H988-10 containing signal peptide
MGWSLILLFLVAVATRVLSQSVQESGPGLVKPSETLSLTCTVSGIDLSSYAISWVRQPPGKGLEYIGYIWNAGNTYYASWAKGRVTISVDTSKNQVDLKLSSVTAADTAVYFCARGTLGDYNGMDPWGPGTLVTVSSASTKGPSVFPLAPSSKSTSGGTAALGCLVKDYFPEPVTVSWNSGALTSGVHTFPAVLQSSGLYSLSSVVTVPSSSLGTQTYICNVNHKPSNTKVDKKVEPKSCDKTHTCPPCPAPELLGGPSVFLFPPKPKDTLMISRTPEVTCVVVDVSHEDPEVKFNWYVDGVEVHNAKTKPREEQYNSTYRVVSVLTVLHQDWLNGKEYKCKVSNKALPAPIEKTISKAKGQPREPQVYTLPPSRDELTKNQVSLTCLVKGFYPSDIAVEWESNGQPENNYKTTPPVLDSDGSFFLYSKLTVDKSRWQQGNVFSCSVMHEALHNHYTQKSLSLSPGK

SEQ ID NO: 22 - protein, 238 aa, Artificial sequence
  Amino acid sequence of the light chain of humanized antibody VEGF165-H988-10 containing signal peptide
MGWSCIILFLVATATGVHSELQLTQSPSSLSASVGDRVTITCQSSQTIYANRRLAWYQQKPGKVPKLLIYGASTLASGVPSRFKGSGSGTDFTLTISSLQPEDVATYYCAGYKSYDGDDVGFGGGTKVEIKRTVAAPSVFIFPPSDEQLKSGTASVVCLLNNFYPREAKVQWKVDNALQSGNSQESVTEQDSKDSTYSLSSTLTLSKADYEKHKVYACEVTHQGLSSPVTKSFNRGEC

SEQ ID NO: 23 - DNA, 354 bp, Artificial sequence
  Nucleotide sequence of the heavy chain variable region of humanized antibody VEGF165-H988-10
cagtctgtccaggagtctggacctggactggtgaagccatctgagaccctgtccctgacttgtactgtgtctggcattgacctgtcctcctatgccatctcctgggtgagacaacctcctggcaagggattggaatacattggctacatctggaatgctggcaacacctactatgcctcctgggctaagggcagggtgaccatctctgtggacaccagcaagaaccaggtggacctgaaactgtcctctgtgacagcagcagacacagcagtctacttctgtgccaggggcaccctgggagactacaatgggatggacccatggggacctggcaccctggtgacagtgtccagc

SEQ ID NO: 24 - DNA, 336 bp, Artificial sequence
  Nucleotide sequence of the light chain variable region of humanized antibody VEGF165-H988-10
gaactccaacttacccagagcccatcctccctgtctgcctctgtgggagacagggtgaccatcacttgtcagtccagccagaccatctatgccaacaggagactggcttggtatcaacagaagcctggcaaggtgccaaaactgctgatttatggagccagcaccctggcatctggagtgccaagcaggttcaagggctctggctctggcacagacttcaccctgaccatctcctccctccaacctgaggatgtggctacctactactgtgctggctacaagtcctatgatggagatgatgtgggctttggaggaggcaccaaggtggagattaag

SEQ ID NO: 25 - protein, 118 aa, Artificial sequence
  Amino acid sequence of the heavy chain variable region of antibody VEGF165-H988-10
QSVQESGPGLVKPSETLSLTCTVSGIDLSSYAISWVRQPPGKGLEYIGYIWNAGNTYYASWAKGRVTISVDTSKNQVDLKLSSVTAADTAVYFCARGTLGDYNGMDPWGPGTLVTVSS

SEQ ID NO: 26 - protein, 112 aa, Artificial sequence
  Amino acid sequence of the light chain variable region of antibody VEGF165-H988-10
ELQLTQSPSSLSASVGDRVTITCQSSQTIYANRRLAWYQQKPGKVPKLLIYGASTLASGVPSRFKGSGSGTDFTLTISSLQPEDVATYYCAGYKSYDGDDVGFGGGTKVEIK

SEQ ID NO: 27 - protein, 13 aa, Oryctolagus cuniculus f. domesticus
QSSKFLWQGRRLA

SEQ ID NO: 28 - protein, 7 aa, Oryctolagus cuniculus f. domesticus
GASTLAS

SEQ ID NO: 29 - protein, 12 aa, Oryctolagus cuniculus f. domesticus
AGYKSYDGDVVG

SEQ ID NO: 30 - protein, 10 aa, Oryctolagus cuniculus f. domesticus
GIDLSSYAIS

SEQ ID NO: 31 - protein, 16 aa, Oryctolagus cuniculus f. domesticus
YIWNDLFTYYASWAKG

SEQ ID NO: 32 - protein, 13 aa, Oryctolagus cuniculus f. domesticus
ARGTLGDYGGMDP

SEQ ID NO: 33 - protein, 448 aa, Artificial sequence
  Amino acid sequence of the heavy chain of humanized antibody VEGF-H988
QSVQESGPGLVKPSETLSLTCTVSGIDLSSYAISWVRQPPGKGLEYIGYIWNDLFTYYASWAKGRVTISVDTSKNQVDLKLSSVTAADTAVYFCARGTLGDYGGMDPWGQGTLVTVSSASTKGPSVFPLAPSSKSTSGGTAALGCLVKDYFPEPVTVSWNSGALTSGVHTFPAVLQSSGLYSLSSVVTVPSSSLGTQTYICNVNHKPSNTKVDKKVEPKSCDKTHTCPPCPAPELLGGPSVFLFPPKPKDTLMISRTPEVTCVVVDVSHEDPEVKFNWYVDGVEVHNAKTKPREEQYNSTYRVVSVLTVLHQDWLNGKEYKCKVSNKALPAPIEKTISKAKGQPREPQVYTLPPSRDELTKNQVSLTCLVKGFYPSDIAVEWESNGQPENNYKTTPPVLDSDGSFFLYSKLTVDKSRWQQGNVFSCSVMHEALHNHYTQKSLSLSPGK

SEQ ID NO: 34 - protein, 219 aa, Artificial sequence
  Amino acid sequence of the light chain of humanized antibody VEGF-H988
ELQLTQSPSSLSASVGDRVTITCQSSKFLWQGRRLAWYQQKPGKVPKLLIYGASTLASGVPSRFKGSGSGTDFTLTISSLQPEDVATYYCAGYKSYDGDVVGFGGGTKVEIKRTVAAPSVFIFPPSDEQLKSGTASVVCLLNNFYPREAKVQWKVDNALQSGNSQESVTEQDSKDSTYSLSSTLTLSKADYEKHKVYACEVTHQGLSSPVTKSFNRGEC

SEQ ID NO: 35 - protein, 467 aa, Artificial sequence
  Amino acid sequence of the heavy chain of humanized antibody VEGF-H988 containing signal peptide
MGWSLILLFLVAVATRVLSQSVQESGPGLVKPSETLSLTCTVSGIDLSSYAISWVRQPPGKGLEYIGYIWNDLFTYYASWAKGRVTISVDTSKNQVDLKLSSVTAADTAVYFCARGTLGDYGGMDPWGQGTLVTVSSASTKGPSVFPLAPSSKSTSGGTAALGCLVKDYFPEPVTVSWNSGALTSGVHTFPAVLQSSGLYSLSSVVTVPSSSLGTQTYICNVNHKPSNTKVDKKVEPKSCDKTHTCPPCPAPELLGGPSVFLFPPKPKDTLMISRTPEVTCVVVDVSHEDPEVKFNWYVDGVEVHNAKTKPREEQYNSTYRVVSVLTVLHQDWLNGKEYKCKVSNKALPAPIEKTISKAKGQPREPQVYTLPPSRDELTKNQVSLTCLVKGFYPSDIAVEWESNGQPENNYKTTPPVLDSDGSFFLYSKLTVDKSRWQQGNVFSCSVMHEALHNHYTQKSLSLSPGK

SEQ ID NO: 36 - protein, 238 aa, Artificial sequence
  Amino acid sequence of the light chain of humanized antibody VEGF-H988 containing signal peptide
MGWSCIILFLVATATGVHSELQLTQSPSSLSASVGDRVTITCQSSKFLWQGRRLAWYQQKPGKVPKLLIYGASTLASGVPSRFKGSGSGTDFTLTISSLQPEDVATYYCAGYKSYDGDVVGFGGGTKVEIKRTVAAPSVFIFPPSDEQLKSGTASVVCLLNNFYPREAKVQWKVDNALQSGNSQESVTEQDSKDSTYSLSSTLTLSKADYEKHKVYACEVTHQGLSSPVTKSFNRGEC

SEQ ID NO: 37 - protein, 19 aa, Artificial sequence
  Amino acid sequence of heavy chain signal peptide
MGWSLILLFLVAVATRVLS

SEQ ID NO: 38 - protein, 19 aa, Artificial sequence
  Amino acid sequence of light chain signal peptide
MGWSCIILFLVATATGVHS

SEQ ID NO: 39 - protein, 118 aa, Artificial sequence
  Amino acid sequence of the heavy chain variable region of humanized antibody VEGF-H988
QSVQESGPGLVKPSETLSLTCTVSGIDLSSYAISWVRQPPGKGLEYIGYIWNDLFTYYASWAKGRVTISVDTSKNQVDLKLSSVTAADTAVYFCARGTLGDYGGMDPWGQGTLVTVSS

SEQ ID NO: 40 - protein, 112 aa, Artificial sequence
  Amino acid sequence of the light chain variable region of humanized antibody VEGF-H988
ELQLTQSPSSLSASVGDRVTITCQSSKFLWQGRRLAWYQQKPGKVPKLLIYGASTLASGVPSRFKGSGSGTDFTLTISSLQPEDVATYYCAGYKSYDGDVVGFGGGTKVEIK

SEQ ID NO: 41 - protein, 330 aa, Homo sapiens [sequence omitted]

SEQ ID NO: 42 - protein, 107 aa, Homo sapiens [sequence omitted]

SEQ ID NO: 43 - DNA, 1404 bp, Artificial sequence
  Nucleotide sequence of humanized antibody VEGF-H988 heavy chain containing signal peptide
atgggctggtccctgattctgctgttcctggtggctgtggctaccagggtgctgagtcagtctgtccaggagtctggacctggactggtgaagccatctgagaccctgtccctgacttgtactgtgtctggcattgacctgtcctcctatgccatctcctgggtgagacaacctcctggcaagggattggaatacattggctacatctggaatgatctcttcacctactatgcctcctgggctaagggcagggtgaccatctctgtggacaccagcaagaaccaggtggacctgaaactgtcctctgtgacagcagcagacacagcagtctacttctgtgccaggggcaccctgggagactacggcgggatggacccatggggacagggcaccctggtgacagtgtccagcgcaagcaccaagggcccatcggtcttccccctggcaccctcctccaagagcacctctgggggcacagcggccctgggctgcctggtcaaggactacttccccgaaccggtgacggtgtcgtggaactcaggcgccctgaccagcggcgtgcacaccttcccggctgtcctacagtcctcaggactctactccctcagcagcgtggtgaccgtgccctccagcagcttgggcacccagacctacatctgcaacgtgaatcacaagcccagcaacaccaaggtggacaagaaagttgagcccaaatcttgtgacaaaactcacacatgcccaccgtgcccagcacctgaactcctggggggaccgtcagtcttcctcttccccccaaaacccaaggacaccctcatgatctcccggacccctgaggtcacgtgcgtggtggtggacgtgagccacgaagaccccgaggtcaagttcaactggtacgtggacggcgtggaggtgcataatgccaagacaaagccgcgggaggagcagtacaacagcacgtaccgtgtggtcagcgtcctcaccgtcctgcaccaggactggctgaatggcaaggagtacaagtgcaaggtctccaacaaagccctcccagcccccatcgagaaaaccatctccaaagccaaagggcagccccgagaaccacaggtgtacaccctgcccccatcccgggatgagctgaccaagaaccaggtcagcctgacctgcctggtcaaaggcttctatcccagcgacatcgccgtggagtgggagagcaatgggcagccggagaacaactacaagaccacgcctcccgtgctggactccgacggctccttcttcctctacagcaagctcaccgtggacaagagcaggtggcagcaggggaacgtcttctcatgctccgtgatgcatgaggctctgcacaaccactacacgcagaagagcctctccctgtctccgggtaaataa

SEQ ID NO: 44 - DNA, 717 bp, Artificial sequence
  Nucleotide sequence of humanized antibody VEGF-H988 light chain containing signal peptide
atgggctggtcctgtatcatcctgttcctggtggctacagccacaggagtgcatagtgaactccaacttacccagagcccatcctccctgtctgcctctgtgggagacagggtgaccatcacttgtcagtccagcaagttcctctggcagggcaggagactggcttggtatcaacagaagcctggcaaggtgccaaaactgctgatttatggagccagcaccctggcatctggagtgccaagcaggttcaagggctctggctctggcacagacttcaccctgaccatctcctccctccaacctgaggatgtggctacctactactgtgctggctacaagtcctatgatggagatgttgtgggctttggaggaggcaccaaggtggagattaagcgtacggtggctgcaccatctgtcttcatcttcccgccatctgatgagcagttgaaatctggaactgcctctgttgtgtgcctgctgaataacttctatcccagagaggccaaagtacagtggaaggtggataacgccctccaatcgggtaactcccaggagagtgtcacagagcaggacagcaaggacagcacctacagcctcagcagcaccctgacgctgagcaaagcagactacgagaaacacaaagtctacgcctgcgaagtcacccatcagggcctgagctcgcccgtcacaaagagcttcaacaggggagagtgttaa

SEQ ID NO: 45 - DNA, 57 bp, Artificial sequence
  Nucleotide sequence of heavy chain signal peptide
atgggctggtccctgattctgctgttcctggtggctgtggctaccagggtgctgagt

SEQ ID NO: 46 - DNA, 57 bp, Artificial sequence
  Nucleotide sequence of light chain signal peptide
atgggctggtcctgtatcatcctgttcctggtggctacagccacaggagtgcatagt

SEQ ID NO: 47 - DNA, 354 bp, Artificial sequence
  Nucleotide sequence of the heavy chain variable region of humanized antibody VEGF-H988
cagtctgtccaggagtctggacctggactggtgaagccatctgagaccctgtccctgacttgtactgtgtctggcattgacctgtcctcctatgccatctcctgggtgagacaacctcctggcaagggattggaatacattggctacatctggaatgatctcttcacctactatgcctcctgggctaagggcagggtgaccatctctgtggacaccagcaagaaccaggtggacctgaaactgtcctctgtgacagcagcagacacagcagtctacttctgtgccaggggcaccctgggagactacggcgggatggacccatggggacagggcaccctggtgacagtgtccagc

SEQ ID NO: 48 - DNA, 336 bp, Artificial sequence
  Nucleotide sequence of the light chain variable region of humanized antibody VEGF-H988
gaactccaacttacccagagcccatcctccctgtctgcctctgtgggagacagggtgaccatcacttgtcagtccagcaagttcctctggcagggcaggagactggcttggtatcaacagaagcctggcaaggtgccaaaactgctgatttatggagccagcaccctggcatctggagtgccaagcaggttcaagggctctggctctggcacagacttcaccctgaccatctcctccctccaacctgaggatgtggctacctactactgtgctggctacaagtcctatgatggagatgttgtgggctttggaggaggcaccaaggtggagattaag

SEQ ID NO: 49 - DNA, 993 bp, Homo sapiens
gcaagcaccaagggcccatcggtcttccccctggcaccctcctccaagagcacctctgggggcacagcggccctgggctgcctggtcaaggactacttccccgaaccggtgacggtgtcgtggaactcaggcgccctgaccagcggcgtgcacaccttcccggctgtcctacagtcctcaggactctactccctcagcagcgtggtgaccgtgccctccagcagcttgggcacccagacctacatctgcaacgtgaatcacaagcccagcaacaccaaggtggacaagaaagttgagcccaaatcttgtgacaaaactcacacatgcccaccgtgcccagcacctgaactcctggggggaccgtcagtcttcctcttccccccaaaacccaaggacaccctcatgatctcccggacccctgaggtcacgtgcgtggtggtggacgtgagccacgaagaccccgaggtcaagttcaactggtacgtggacggcgtggaggtgcataatgccaagacaaagccgcgggaggagcagtacaacagcacgtaccgtgtggtcagcgtcctcaccgtcctgcaccaggactggctgaatggcaaggagtacaagtgcaaggtctccaacaaagccctcccagcccccatcgagaaaaccatctccaaagccaaagggcagccccgagaaccacaggtgtacaccctgcccccatcccgggatgagctgaccaagaaccaggtcagcctgacctgcctggtcaaaggcttctatcccagcgacatcgccgtggagtgggagagcaatgggcagccggagaacaactacaagaccacgcctcccgtgctggactccgacggctccttcttcctctacagcaagctcaccgtggacaagagcaggtggcagcaggggaacgtcttctcatgctccgtgatgcatgaggctctgcacaaccactacacgcagaagagcctctccctgtctccgggtaaataa

SEQ ID NO: 50 - DNA, 324 bp, Homo sapiens
cgtacggtggctgcaccatctgtcttcatcttcccgccatctgatgagcagttgaaatctggaactgcctctgttgtgtgcctgctgaataacttctatcccagagaggccaaagtacagtggaaggtggataacgccctccaatcgggtaactcccaggagagtgtcacagagcaggacagcaaggacagcacctacagcctcagcagcaccctgacgctgagcaaagcagactacgagaaacacaaagtctacgcctgcgaagtcacccatcagggcctgagctcgcccgtcacaaagagcttcaacaggggagagtgttaa

SEQ ID NO: 51 - protein, 246 aa, Artificial sequence
  Amino acid sequence of the rabbit antibody scFv used in the construction of antibody VEGF165-R988
ELDLTQTPSPVSAAVGGTVTINCQSSQTIYANRRLAWYQQKPGQPPKLLIYGASTLASGVPSRFKGSGSGTQFTLTISGVQCDDAATYYCAGYKSYDGDDVGFGGGTEVVVKSSGGGGSGGGGGGSSRSSQSVEESGGRLVTPGTPLTLTCTVSGIDLSSYAISWVRQAPGKGLEYIGYIWNAGNTYYASWAKGRFTISKTSTTVDLKITSPTTEDTATYFCARGTLGDYNGMDPWGPGTLVTVSS

SEQ ID NO: 52 - protein, 18 aa, Artificial sequence
  Amino acid sequence of the linker used in the construction of the phage antibody library for the linkage of rabbit antibody scFv
SSGGGGSGGGGGGSSRSS

SEQ ID NO: 53 - DNA, 1377 bp, Artificial sequence
  Nucleotide sequence of rabbit antibody VEGF165-R988 heavy chain containing signal peptide
atgggctggtccctgattctgctgttcctggtggctgtggctaccagggtgctgagtcagtcggtggaggagtccgggggtcgcctggtaacgcctgggacacccctgacactcacctgcacagtctctggaatcgacctcagtagctatgcaataagctgggtccgccaggctccagggaaggggctggaatacatcggatacatttggaatgctggtaacacctactacgcgagctgggcaaaaggccgattcaccatctccaaaacctcgaccacggtggatctgaaaatcaccagtccgacaaccgaggacacggccacctatttctgtgccagaggaacattaggggactacaatggcatggacccctggggcccagggaccctcgtcaccgtctcttcaggtcaacctaaggctccgtcagtcttcccactggccccctgctgcggggacacacccagctccacggtgaccctgggctgcctggtcaaaggctacctcccggagccagtgaccgtgacctggaactcgggcaccctcaccaatggggtacgcaccttcccgtccgtccggcagtcctcaggcctctactcgctgagcagcgtggtgagcgtgacctcaagcagccagcccgtcacctgcaacgtggcccacccagccaccaacaccaaagtggacaagaccgttgcgccctcgacatgcagcaagcccacgtgcccaccccctgaactcctggggggaccgtctgtcttcatcttccccccaaaacccaaggacaccctcatgatctcacgcacccccgaggtcacatgcgtggtggtggacgtgagccaggatgaccccgaggtgcagttcacatggtacataaacaacgagcaggtgcgcaccgcccggccgccgctacgggagcagcagttcaacagcacgatccgcgtggtcagcaccctccccatcgcgcaccaggactggctgaggggcaaggagttcaagtgcaaagtccacaacaaggcactcccggcccccatcgagaaaaccatctccaaagccagagggcagcccctggagccgaaggtctacaccatgggccctccccgggaggagctgagcagcaggtcggtcagcctgacctgcatgatcaacggcttctacccttccgacatctcggtggagtgggagaagaacgggaaggcagaggacaactacaagaccacgccggccgtgctggacagcgacggctcctacttcctctacagcaagctctcagtgcccacgagtgagtggcagcggggcgacgtcttcacctgctccgtgatgcacgaggccttgcacaaccactacacgcagaagtccatctcccgctctccgggtaaataa

SEQ ID NO: 54 - DNA, 708 bp, Artificial sequence
  Nucleotide sequence of the rabbit antibody VEGF165-R988 light chain containing signal peptide
atgggctggtcctgtatcatcctgttcctggtggctacagccacaggagtgcatagtgagctcgatctgacccagactccatcccccgtgtctgcggctgttggaggcacagtcaccatcaattgccagtccagtcagactatttatgctaacaggcgcttagcctggtatcaacagaaaccagggcagcctcccaagctcctgatctatggtgcatccactctggcatctggggtcccatcgcggttcaaaggcagtggatctgggacacagttcactctcaccatcagcggcgtgcagtgtgacgatgctgccacttactactgtgcaggctataaaagttatgatggtgatgatgttggtttcggcggagggaccgaggtggtcgtcaaaggggatccagttgcacctactgtcctcatcttcccaccagctgctgatcaggtggcaactggaacagtcaccatcgtgtgtgtggcgaataaatactttcccgatgtcaccgtcacctgggaggtggatggcaccacccaaacaactggcatcgagaacagtaaaacaccgcagaattctgcagattgtacctacaacctcagcagcactctgacactgaccagcacacagtacaacagccacaaagagtacacctgcaaggtgacccagggcacgacctcagtcgtccagagcttcaataggggtgactgttaa

SEQ ID NO: 55 - protein, 458 aa, Artificial sequence
  Amino acid sequence of the rabbit antibody VEGF165-R988 heavy chain containing signal peptide
MGWSLILLFLVAVATRVLSQSVEESGGRLVTPGTPLTLTCTVSGIDLSSYAISWVRQAPGKGLEYIGYIWNAGNTYYASWAKGRFTISKTSTTVDLKITSPTTEDTATYFCARGTLGDYNGMDPWGPGTLVTVSSGQPKAPSVFPLAPCCGDTPSSTVTLGCLVKGYLPEPVTVTWNSGTLTNGVRTFPSVRQSSGLYSLSSVVSVTSSSQPVTCNVAHPATNTKVDKTVAPSTCSKPTCPPPELLGGPSVFIFPPKPKDTLMISRTPEVTCVVVDVSQDDPEVQFTWYINNEQVRTARPPLREQQFNSTIRVVSTLPIAHQDWLRGKEFKCKVHNKALPAPIEKTISKARGQPLEPKVYTMGPPREELSSRSVSLTCMINGFYPSDISVEWEKNGKAEDNYKTTPAVLDSDGSYFLYSKLSVPTSEWQRGDVFTCSVMHEALHNHYTQKSISRSPGK

SEQ ID NO: 56 - protein, 235 aa, Artificial sequence
  Amino acid sequence of the rabbit antibody VEGF165-R988 light chain containing signal peptide
MGWSCIILFLVATATGVHSELDLTQTPSPVSAAVGGTVTINCQSSQTIYANRRLAWYQQKPGQPPKLLIYGASTLASGVPSRFKGSGSGTQFTLTISGVQCDDAATYYCAGYKSYDGDDVGFGGGTEVVVKGDPVAPTVLIFPPAADQVATGTVTIVCVANKYFPDVTVTWEVDGTTQTTGIENSKTPQNSADCTYNLSSTLTLTSTQYNSHKEYTCKVTQGTTSVVQSFNRGDC

SEQ ID NO: 57 - protein, 323 aa, Oryctolagus cuniculus f. domesticus
GQPKAPSVFPLAPCCGDTPSSTVTLGCLVKGYLPEPVTVTWNSGTLTNGVRTFPSVRQSSGLYSLSSVVSVTSSSQPVTCNVAHPATNTKVDKTVAPSTCSKPTCPPPELLGGPSVFIFPPKPKDTLMISRTPEVTCVVVDVSQDDPEVQFTWYINNEQVRTARPPLREQQFNSTIRVVSTLPIAHQDWLRGKEFKCKVHNKALPAPIEKTISKARGQPLEPKVYTMGPPREELSSRSVSLTCMINGFYPSDISVEWEKNGKAEDNYKTTPAVLDSDGSYFLYSKLSVPTSEWQRGDVFTCSVMHEALHNHYTQKSISRSPGK

SEQ ID NO: 58 - protein, 104 aa, Oryctolagus cuniculus f. domesticus
GDPVAPTVLIFPPAADQVATGTVTIVCVANKYFPDVTVTWEVDGTTQTTGIENSKTPQNSADCTYNLSSTLTLTSTQYNSHKEYTCKVTQGTTSVVQSFNRGDC

SEQ ID NO: 59 - DNA, 33 bp, Artificial sequence
  Forward primer F1 for amplifying the heavy chain variable region
accagggtgctgagtcagtcggtggaggagtcc

SEQ ID NO: 60 - DNA, 24 bp, Artificial sequence
  Reverse primer R1 for amplifying the heavy chain variable region
tgtgaccagggtacctgggcccca

SEQ ID NO: 61 - DNA, 35 bp, Artificial sequence
  Forward primer F2 for amplifying the light chain variable region
acaggagtgcatagtgagctcgatctgacccagac

SEQ ID NO: 62 - DNA, 35 bp, Artificial sequence
  Reverse primer R2 for amplifying the light chain variable region
ggtgcaactggatcccctttgacgaccacctcggt

SEQ ID NO: 63 - DNA, 50 bp, Artificial sequence
  Forward primer F3 for whole gene synthesis of the heavy chain variable region
ccacaggagtgcatagtgaactccaacttacccagagcccatcctccctg

SEQ ID NO: 64 - DNA, 33 bp, Artificial sequence
  Reverse primer R3 for whole gene synthesis of the heavy chain variable region
cctgtctcccacagaggcagacagggaggatgg

SEQ ID NO: 65 - DNA, 33 bp, Artificial sequence
  Forward primer F4 for whole gene synthesis of the heavy chain variable region
tctgtgggagacagggtgaccatcacttgtcag

SEQ ID NO: 66 - DNA, 33 bp, Artificial sequence
  Reverse primer R4 for whole gene synthesis of the heavy chain variable region
ggcatagatggtctggctggactgacaagtgat

SEQ ID NO: 67 - DNA, 28 bp, Artificial sequence
  Forward primer F5 for whole gene synthesis of the heavy chain variable region
cagaccatctatgccaacaggagactgg

SEQ ID NO: 68 - DNA, 28 bp, Artificial sequence
  Reverse primer R5 for whole gene synthesis of the heavy chain variable region
ttctgttgataccaagccagtctcctgt

SEQ ID NO: 69 - DNA, 28 bp, Artificial sequence
  Forward primer F6 for whole gene synthesis of the heavy chain variable region
ttggtatcaacagaagcctggcaaggtg

SEQ ID NO: 70 - DNA, 28 bp, Artificial sequence
  Reverse primer R6 for whole gene synthesis of the heavy chain variable region
aaatcagcagttttggcaccttgccagg

SEQ ID NO: 71 - DNA, 28 bp, Artificial sequence
  Forward primer F7 for whole gene synthesis of the heavy chain variable region
caaaactgctgatttatggagccagcac

SEQ ID NO: 72 - DNA, 28 bp, Artificial sequence
  Reverse primer R7 for whole gene synthesis of the heavy chain variable region
cactccagatgccagggtgctggctcca

SEQ ID NO: 73 - DNA, 33 bp, Artificial sequence
  Forward primer F8 for whole gene synthesis of the heavy chain variable region
ctggcatctggagtgccaagcaggttcaagggc

SEQ ID NO: 74 - DNA, 33 bp, Artificial sequence
  Reverse primer R8 for whole gene synthesis of the heavy chain variable region
gaagtctgtgccagagccagagcccttgaacct

SEQ ID NO: 75 - DNA, 33 bp, Artificial sequence
  Forward primer F9 for whole gene synthesis of the heavy chain variable region
tctggcacagacttcaccctgaccatctcctcc

SEQ ID NO: 76 - DNA, 33 bp, Artificial sequence
  Reverse primer R9 for whole gene synthesis of the heavy chain variable region
agccacatcctcaggttggagggaggagatggt

SEQ ID NO: 77 - DNA, 33 bp, Artificial sequence
  Forward primer F10 for whole gene synthesis of the heavy chain variable region
cctgaggatgtggctacctactactgtgctggc

SEQ ID NO: 78 - DNA, 33 bp, Artificial sequence
  Reverse primer R10 for whole gene synthesis of the heavy chain variable region
atctccatcataggacttgtagccagcacagta

SEQ ID NO: 79 - DNA, 33 bp, Artificial sequence
  Forward primer F11 for whole gene synthesis of the heavy chain variable region
tcctatgatggagatgatgtgggctttggagga

SEQ ID NO: 80 - DNA, 50 bp, Artificial sequence
  Reverse primer R11 for whole gene synthesis of the heavy chain variable region
ggtgcagccaccgtacgcttaatctccaccttggtgcctcctccaaagcc

SEQ ID NO: 81 - DNA, 51 bp, Artificial sequence
  Forward primer F12 for whole gene synthesis of the light chain variable region
gctaccagggtgctgagtcagtctgtccaggagtctggacctggactggtg

SEQ ID NO: 82 - DNA, 33 bp, Artificial sequence
  Reverse primer R12 for whole gene synthesis of the light chain variable region
ggacagggtctcagatggcttcaccagtccagg

SEQ ID NO: 83 - DNA, 33 bp, Artificial sequence
  Forward primer F13 for whole gene synthesis of the light chain variable region
tctgagaccctgtccctgacttgtactgtgtct

SEQ ID NO: 84 - DNA, 33 bp, Artificial sequence
  Reverse primer R13 for whole gene synthesis of the light chain variable region
ataggaggacaggtcaatgccagacacagtaca

SEQ ID NO: 85 - DNA, 31 bp, Artificial sequence
  Forward primer F14 for whole gene synthesis of the light chain variable region
gacctgtcctcctatgccatctcctgggtga

SEQ ID NO: 86 - DNA, 31 bp, Artificial sequence
  Reverse primer R14 for whole gene synthesis of the light chain variable region
cccttgccaggaggttgtctcacccaggaga

SEQ ID NO: 87 - DNA, 31 bp, Artificial sequence
  Forward primer F15 for whole gene synthesis of the light chain variable region
acctcctggcaagggattggaatacattggc

SEQ ID NO: 88 - DNA, 31 bp, Artificial sequence
  Reverse primer R15 for whole gene synthesis of the light chain variable region
tgccagcattccagatgtagccaatgtattc

SEQ ID NO: 89 - DNA, 31 bp, Artificial sequence
  Forward primer F16 for whole gene synthesis of the light chain variable region
tctggaatgctggcaacacctactatgcctc

SEQ ID NO: 90 - DNA, 31 bp, Artificial sequence
  Reverse primer R16 for whole gene synthesis of the light chain variable region
caccctgcccttagcccaggaggcatagtag

SEQ ID NO: 91 - DNA, 33 bp, Artificial sequence
  Forward primer F17 for whole gene synthesis of the light chain variable region
gctaagggcagggtgaccatctctgtggacacc

SEQ ID NO: 92 - DNA, 33 bp, Artificial sequence
  Reverse primer R17 for whole gene synthesis of the light chain variable region
caggtccacctggttcttgctggtgtccacaga

SEQ ID NO: 93 - DNA, 33 bp, Artificial sequence
  Forward primer F18 for whole gene synthesis of the light chain variable region
aaccaggtggacctgaaactgtcctctgtgaca

SEQ ID NO: 94 - DNA, 33 bp, Artificial sequence
  Reverse primer R18 for whole gene synthesis of the light chain variable region
gtagactgctgtgtctgctgctgtcacagagga

SEQ ID NO: 95 - DNA, 33 bp, Artificial sequence
  Forward primer F19 for whole gene synthesis of the light chain variable region
gacacagcagtctacttctgtgccaggggcacc

SEQ ID NO: 96 - DNA, 33 bp, Artificial sequence
  Reverse primer R19 for whole gene synthesis of the light chain variable region
catcccattgtagtctcccagggtgcccctggc

SEQ ID NO: 97 - DNA, 33 bp, Artificial sequence
  Forward primer F20 for whole gene synthesis of the light chain variable region
gactacaatgggatggacccatggggacctggc

SEQ ID NO: 98 - DNA, 50 bp, Artificial sequence
  Reverse primer R20 for whole gene synthesis of the light chain variable region
gggcccttggtgctagcgctggacactgtcaccagggtgccaggtcccca